European Patent Application EP 4 527 399 A1, published March 26, 2025. Title: Composition for the Treatment of Tinea. Applicant: マルホ株式会社. The sequence listing filed with the application follows.

SEQUENCE LISTING (21 sequences)

SEQ ID NO: 1 - DNA, 1268 bp, Staphylococcus hominis
  source 1..1268: mol_type = genomic DNA
agcttgctcctttgacgttagcggcggacgggtgagtaacacgtgggtaacctacctataagactgggataacttcgggaaaccggagctaataccggataatatttcgaaccgcatggttcgatagtgaaagatggctttgctatcacttatagatggacctgcgccgtattagctagttggtaaggtaacggcttaccaaggcaacgatacgtagccgacctgagagggtgatcggccacactggaactgagacacggtccagactcctacgggaggcagcagtagggaatcttccgcaatgggcgaaagcctgacggagcaacgccgcgtgagtgatgaaggtcttcggatcgtaaaactctgttattagggaagaacaaacgtgtaagtaactgtgcacgtcttgacggtacctaatcagaaagccacggctaactacgtgccagcagccgcggtaatacgtaggtggcaagcgttatccggaattattgggcgtaaagcgcgcgtaggcggttttttaagtctgatgtgaaagcccacggctcaaccgtggagggtcattggaaactggaaaacttgagtgcagaagaggaaagtggaattccatgtgtagcggtgaaatgcgcagagatatggaggaacaccagtggcgaaggcgactttctggtctgtaactgacgctgatgtgcgaaagcgtggggatcaaacaggattagataccctggtagtccacgccgtaaacgatgagtgctaagtgttagggggtttccgccccttagtgctgcagctaacgcattaagcactccgcctggggagtacgaccgcaaggttgaaactcaaaggaattgacggggacccgcacaagcggtggagcatgtggtttaattcgaagcaacgcgaagaaccttaccaaatcttgacatcctttgacccttctagagatagaagtttccccttcgggggacaaagtgacaggtggtgcatggttgtcgtcagctcgtgtcgtgagatgttgggttaagtcccgcaacgagcgcaacccttaagcttagttgccatcattaagttgggcactctaagttgactgccggtgacaaaccggaggaaggtggggatgacgtcaaatcatcatgccccttatgatttgggctacacacgtgctacaatggacaatacaaagggcagcgaaaccgcgaggtcaagcaaatcccataaagttgttctcagttcggattgtagtctgcaactcgactacatgaagctgg

SEQ ID NO: 2 - DNA, 1268 bp, Staphylococcus hominis
  source 1..1268: mol_type = genomic DNA
agcttgctcctttgacgttagcggcggacgggtgagtaacacgtgggtaacctacctataagactgggataacttcgggaaaccggagctaataccggataatatttcgaaccgcatggttcgatagtgaaagatggccctgctatcacttatagatggacctgcgccgtattagctagttggtaaggtaacggcttaccaaggcaacgatacgtagccgacctgagagggtgatcggccacactggaactgagacacggtccagactcctacgggaggcagcagtagggaatcttccgcaatgggcgaaagcctgacggagcaacgccgcgtgagtgatgaaggtcttcggatcgtaaaactctgttattagggaagaacaaacgtgtaagtaactgtgcacgtcttgacggtacctaatcagaaagccacggctaactacgtgccagcagccgcggtaatacgtaggtggcaagcgttatccggaattattgggcgtaaagcgcgcgtaggcggttttttaagtctgatgtgaaagcccacggctcaaccgtggagggtcattggaaactggaaaacttgagtgcagaagaggaaagtggaattccatgtgtagcggtgaaatgcgcagagatatggaggaacaccagtggcgaaggcgactttctggtctgtaactgacgctgatgtgcgaaagcgtggggatcaaacaggattagataccctggtagtccacgccgtaaacgatgagtgctaagtgttagggggtttccgccccttagtgctgcagctaacgcattaagcactccgcctggggagtacgaccgcaaggttgaaactcaaaggaattgacggggacccgcacaagcggtggagcatgtggtttaattcgaagcaacgcgaagaaccttaccaaatcttgacatcctttgacccttctagagatagaagtttccccttcgggggacaaagtgacaggtggtgcatggttgtcgtcagctcgtgtcgtgagatgttgggttaagtcccgcaacgagcgcaacccttaagcttagttgccatcattaagttgggcactctaagttgactgccggtgacaaaccggaggaaggtggggatgacgtcaaatcatcatgccccttatgatttgggctacacacgtgctacaatggacaatacaaagggcagcgaaaccgcgaggtcaagcaaatcccataaagttgttctcagttcggattgtagtctgcaactcgactacatgaagctgg

SEQ ID NO: 3 - DNA, 1268 bp, Staphylococcus hominis
  source 1..1268: mol_type = genomic DNA
agcttgctcctttgacgttagcggcggacgggtgagtaacacgtgggtaacctacctataagactgggataacttcgggaaaccggagctaataccggataatatttcgaaccgcatggttcgatagtgaaagatggctttgctatcacttatagatggacctgcgccgtattagctagttggtaaggtaacggcttaccaaggcaacgatacgtagccgacctgagagggtgatcggccacactggaactgagacacggtccagactcctacgggaggcagcagtagggaatcttccgcaatgggcgaaagcctgacggagcaacgccgcgtgagtgatgaaggtcttcggatcgtaaaactctgttattagggaagaacaaacgtgtaagtaactgtgcacgtcttgacggtacctaatcagaaagccacggctaactacgtgccagcagccgcggtaatacgtaggtggcaagcgttatccggaattattgggcgtaaagcgcgcgtaggcggttttttaagtctgatgtgaaagcccacggctcaaccgtggagggtcattggaaactggaaaacttgagtgcagaagaggaaagtggaattccatgtgtagcggtgaaatgcgcagagatatggaggaacaccagtggcgaaggcgactttctggtctgtaactgacgctgatgtgcgaaagcgtggggatcaaacaggattagataccctggtagtccacgccgtaaacgatgagtgctaagtgttagggggtttccgccccttagtgctgcagctaacgcattaagcactccgcctggggagtacgaccgcaaggttgaaactcaaaggaattgacggggacccgcacaagcggtggagcatgtggtttaattcgaagcaacgcgaagaaccttaccaaatcttgacatcctttgacccttctagagatagaagtttccccttcgggggacaaagtgacaggtggtgcatggttgtcgtcagctcgtgtcgtgagatgttgggttaagtcccgcaacgagcgcaacccttaagcttagttgccatcattaagttgggcactctaagttgactgccggtgacaaaccggaggaaggtggggatgacgtcaaatcatcatgccccttatgatttgggctacacacgtgctacaatggacaatacaaagggcagcgaaaccgcgaggtcaagcaaatcccataaagttgttctcagttcggattgtagtctgcaactcgactacatgaagttgg

SEQ ID NO: 4 - DNA, 1268 bp, Staphylococcus hominis
  source 1..1268: mol_type = genomic DNA
agcttgctcctttgacgttagcggcggacgggtgagtaacacgtgggtaacctacctataagactgggataacttcgggaaaccggagctaataccggataatatttcgaaccgcatggttcgatagtgaaagatggctctgctatcacttatagatggacctgcgccgtattagctagttggtaaggtaacggcttaccaaggcaacgatacgtagccgacctgagagggtgatcggccacactggaactgagacacggtccagactcctacgggaggcagcagtagggaatcttccgcaatgggcgaaagcctgacggagcaacgccgcgtgagtgatgaaggtcttcggatcgtaaaactctgttattagggaagaacaaacgtgtaagtaactgtgcacgtcttgacggtacctaatcagaaagccacggctaactacgtgccagcagccgcggtaatacgtaggtggcaagcgttatccggaattattgggcgtaaagcgcgcgtaggcggttttttaagtctgatgtgaaagcccacggctcaaccgtggagggtcattggaaactggaaaacttgagtgcagaagaggaaagtggaattccatgtgtagcggtgaaatgcgcagagatatggaggaacaccagtggcgaaggcgactttctggtctgtaactgacgctgatgtgcgaaagcgtggggatcaaacaggattagataccctggtagtccacgccgtaaacgatgagtgctaagtgttagggggtttccgccccttagtgctgcagctaacgcattaagcactccgcctggggagtacgaccgcaaggttgaaactcaaaggaattgacggggacccgcacaagcggtggagcatgtggtttaattcgaagcaacgcgaagaaccttaccaaatcttgacatcctttgacccttctagagatagaagtttccccttcgggggacaaagtgacaggtggtgcatggttgtcgtcagctcgtgtcgtgagatgttgggttaagtcccgcaacgagcgcaacccttaagcttagttgccatcattaagttgggcactctaagttgactgccggtgacaaaccggaggaaggtggggatgacgtcaaatcatcatgccccttatgatttgggctacacacgtgctacaatggacaatacaaagggcagcgaaaccgcgaggtcaagcaaatcccataaagttgttctcagttcggattgtagtctgcaactcgactacatgaagctgg

SEQ ID NO: 5 - DNA, 1268 bp, Staphylococcus hominis
  source 1..1268: mol_type = genomic DNA
agcttgctcctttgacgttagcggcggacgggtgagtaacacgtaggtaacctacctataagactgggataacttcgggaaaccggagctaataccggataatatttcgaaccgcatggttcgatagtgaaagatggctttgctatcacttatagatggacctgcgccgtattagctagttggtaaggtaacggcttaccaaggcaacgatacgtagccgacctgagagggtgatcggccacactggaactgagacacggtccagactcctacgggaggcagcagtagggaatcttccgcaatgggcgaaagcctgacggagcaacgccgcgtgagtgatgaaggtcttcggatcgtaaaactctgttattagggaagaacaaacgtgtaagtaactgtgcacgtcttgacggtacctaatcagaaagccacggctaactacgtgccagcagccgcggtaatacgtaggtggcaagcgttatccggaattattgggcgtaaagcgcgcgtaggcggttttttaagtctgatgtgaaagcccacggctcaaccgtggagggtcattggaaactggaaaacttgagtgcagaagaggaaagtggaattccatgtgtagcggtgaaatgcgcagagatatggaggaacaccagtggcgaaggcgactttctggtctgtaactgacgctgatgtgcgaaagcgtggggatcaaacaggattagataccctggtagtccacgccgtaaacgatgagtgctaagtgttagggggtttccgccccttagtgctgcagctaacgcattaagcactccgcctggggagtacgaccgcaaggttgaaactcaaaggaattgacggggacccgcacaagcggtggagcatgtggtttaattcgaagcaacgcgaagaaccttaccaaatcttgacatcctttgacccttctagagatagaagtttccccttcgggggacaaagtgacaggtggtgcatggttgtcgtcagctcgtgtcgtgagatgttgggttaagtcccgcaacgagcgcaacccttaagcttagttgccatcattaagttgggcactctaagttgactgccggtgacaaaccggaggaaggtggggatgacgtcaaatcatcatgccccttatgatttgggctacacacgtgctacaatggacaatacaaagggcagcgaaaccgcgaggtcaagcaaatcccataaagttgttctcagttcggattgtagtctgcaactcgactacatgaagctgg

SEQ ID NO: 6 - DNA, 1268 bp, Staphylococcus hominis
  source 1..1268: mol_type = genomic DNA
agcttgctcctttgacgttagcggcggacgggtgagtaacacgtaggtaacctacctataagactgggataacttcgggaaaccggagctaataccggataatatttcgaaccgcatggttcgatagtgaaagatggctttgctatcacttatagatggacctgcgccgtattagctagttggtaaggtaacggcttaccaaggcaacgatacgtagccgacctgagagggtgatcggccacactggaactgagacacggtccagactcctacgggaggcagcagtagggaatcttccgcaatgggcgcaagcctgacggagcaacgccgcgtgagtgatgaaggtcttcggatcgtaaaactctgttattagggaagaacaaacgtgtaagtaactgtgcacgtcttgacggtacctaatcagaaagccacggctaactacgtgccagcagccgcggtaatacgtaggtggcaagcgttatccggaattattgggcgtaaagcgcgcgtaggcggttttttaagtctgatgtgaaagcccacggctcaaccgtggagggtcattggaaactggaaaacttgagtgcagaagaggaaagtggaattccatgtgtagcggtgaaatgcgcagagatatggaggaacaccagtggcgaaggcgactttctggtctgtaactgacgctgatgtgcgaaagcgtggggatcaaacaggattagataccctggtagtccacgccgtaaacgatgagtgctaagtgttagggggtttccgccccttagtgctgcagctaacgcattaagcactccgcctggggagtacgaccgcaaggttgaaactcaaaggaattgacggggacccgcacaagcggtggagcatgtggtttaattcgaagcaacgcgaagaaccttaccaaatcttgacatcctttgacccttctagagatagaagtttccccttcgggggacaaagtgacaggtggtgcatggttgtcgtcagctcgtgtcgtgagatgttgggttaagtcccgcaacgagcgcaacccttaagcttagttgccatcattaagttgggcactctaagttgactgccggtgacaaaccggaggaaggtggggatgacgtcaaatcatcatgccccttatgatttgggctacacacgtgctacaatggacaatacaaagggcagcgaaaccgcgaggtcaagcaaatcccataaagttgttctcagttcggattgtagtctgcaactcgactacatgaagctgg

SEQ ID NO: 7 - DNA, 1267 bp, Staphylococcus hominis
  source 1..1267: mol_type = genomic DNA
agcttgctcctttgacgttagcggcggacgggtgagtaacacgtaggtaacctacctataagactgggataacttcgggaaaccggagctaataccggataatatttcgaaccgcatggttcgatagtgaaagatggctttgctatcacttatagatggacctgcgccgtattagctagttggtaaggtaacggcttaccaaggcaacgatacgtagccgacctgagagggtgatcggccacactggaactgagacacggtccagactcctacgggaggcagcagtagggaatcttccgcaatgggcgaaagcctgacggagcaacgccgcgtgagtgatgaaggtcttcggatcgtaaaactctgttattagggaagaacaaacgtgtaagtaactgtgcacgtcttgacggtacctaatcagaaagccacggctaactacgtgccagcagccgcggtaatacgtaggtggcaagcgttatccggattattgggcgtaaagcgcgcgtaggcggttttttaagtctgatgtgaaagcccacggctcaaccgtggagggtcattggaaactggaaaacttgagtgcagaagaggaaagtggaattccatgtgtagcggtgaaatgcgcagagatatggaggaacaccagtggcgaaggcgactttctggtctgtaactgacgctgatgtgcgaaagcgtggggatcaaacaggattagataccctggtagtccacgccgtaaacgatgagtgctaagtgttagggggtttccgccccttagtgctgcagctaacgcattaagcactccgcctggggagtacgaccgcaaggttgaaactcaaaggaattgacggggacccgcacaagcggtggagcatgtggtttaattcgaagcaacgcgaagaaccttaccaaatcttgacatcctttgacccttctagagatagaagtttccccttcgggggacaaagtgacaggtggtgcatggttgtcgtcagctcgtgtcgtgagatgttgggttaagtcccgcaacgagcgcaacccttaagcttagttgccatcattaagttgggcactctaagttgactgccggtgacaaaccggaggaaggtggggatgacgtcaaatcatcatgccccttatgatttgggctacacacgtgctacaatggacaatacaaagggcagcgaaaccgcgaggtcaagcaaatcccataaagttgttctcagttcggattgtagtctgcaactcgactacatgaagctgg

SEQ ID NO: 8 - DNA, 1269 bp, Staphylococcus hominis
  source 1..1269: mol_type = genomic DNA
agcttgctcctttgacgttagcggcggacgggtgagtaacacgtaggtaacctacctataagactgggataacttcgggaaaccggagctaataccggataatatttcgaaccgcatggttcgatagtgaaagatggctttgctatcacttatagatggacctgcgccgtattagctagttggtaaggtaacggcttaccaaggcaacgatacgtagccgacctgagagggtgatcggccacactggaactgagacacggtccagactcctacgggaggcagcagtagggaatcttccgcaatgggcgaaagcctgacggagcaacgccgcgtgagtgatgaaggtcttcggatcgtaaaactctgttattagggaagaacaaacgtgtaagtaactgtgcacgtcttgacggtacctaatcagaaagccacggctaactacgtgccagcagccgcggtaatacgtaggtggcaagcgttatccggaattattgggcgtaaagcgcgcgtaggcggttttttaagtctgatgtgaaagcccacggctcaaccgtggagggtcattggaaactggaaaacttgagtgcagaagaggaaagtggaattccatgtgtagcggtgaaatgcgcagagatatggaggaacaccagtggcgaaggcgactttctggtctgtaactgacgctgatgtgcgaaagcgtggggatcaaacaggattagataccctggtagtccacgccgtaaacgatgagtgctaagtgttagggggtttccgccccttagtgctgcagctaacgcattaagcactccgcctggggagtacgaccgcaaggttgaaactcaaaggaattgacggggacccgcacaagcggtggagcatgtggtttaattcgaagcaacgcgaagaaccttaccaaatcttgacatcctttgacccttctagagatagaagtttccccttcgggggacaaagtgacaggtggtgcatggttgtcgtcagctcgtgtcgtgagatgttgggttaagtcccgcaacgagcgcaacccttaagcttagttgccatcattaagttgggcactctaagttgactgccggtgacaaaccggaggaaggtggggatgacgtcaaatcatcatgccccttatgatttgggctacacacgtgctacaatggacaatacaaaagggcagcgaaaccgcgaggtcaagcaaatcccataaagttgttctcagttcggattgtagtctgcaactcgactacatgaagctgg

SEQ ID NO: 9 - DNA, 1269 bp, Staphylococcus hominis
  source 1..1269: mol_type = genomic DNA
agcttgctcctttgacgttagcggcggacgggtgagtaacacgtaggtaacctacctataagactgggataacttcgggaaaccggagctaataccggataatatttcgaaccgcatggttcgatagtgaaagatggctttgctatcacttatagatggacctgcgccgtattagctagttggtaaggtaacggcttaccaaggcaacgatacgtagccgacctgagagggtgatcggccacactggaactgagacacggtccagactcctacgggaggcagcagtagggaatcttccgcaatgggcgaaagcctgacggagcaacgccgcgtgagtgatgaaggtcttcggatcgtaaaactctgttattagggaagaacaaacgtgtaagtaactgtgcacgtcttgacggtacctaatcagaaagccacggctaactacgtgccagcagccgcggtaatacgtaggtggcaagcgttatccggaattattgggcgtaaagcgcgcgtaggcggttttttaagtctgatgtgaaagcccacggctcaaccgtggagggtcattggaaactggaaaacttgagtgcagaagaggaaagtggaattccatgtgtagcggtgaaatgcgcagagatatggaggaacaccagtggcgaaggcgactttctggtctgtaactgacgctgatgtgcgaaagcgtggggatcaaacaggattagataccctggtagtccacgccgtaaacgatgagtgctaagtgttagggggtttccgccccttagtgctgcagctaacgcattaagcactccgcctggggagtacgaccgcaaggttgaaactcaaaggaattgacggggacccgcacaagcggtggagcatgtggtttaattcgaagcaacgcgaagaaccttaccaaatcttgacatcctttgacccttctagagatagaagtttccccttcgggggacaaagtgacaggtggtgcatggttgtcgtcagctcgtgtcgtgagatgttgggttaagtcccgcaacgagcgcaacccttaagcttagttgccatcattaagttgggcactctaagttgactgccggtgacaaaccggaggaaggtggggatgacgtcaaatcatcatgccccttatgatttgggctacacacgtgctacaatggacaatacaaagggcagcgaaaccgcgaggtcaagcaaatcccataaagttgttctcagttcgggattgtagtctgcaactcgactacatgaagctgg

SEQ ID NO: 10 - DNA, 1268 bp, Staphylococcus haemolyticus
  source 1..1268: mol_type = genomic DNA
agcttgctcctttgacgttagcggcggacgggtgagtaacacgtgggtaacctacctataagactgggataacttcgggaaaccggagctaataccggataatatttcgaaccgcatggttcgatagtgaaagatggttttgctatcacttatagatggacccgcgccgtattagctagttggtaaggtaacggcttaccaaggcgacgatacgtagccgacctgagagggtgatcggccacactggaactgagacacggtccagactcctacgggaggcagcagtagggaatcttccgcaatgggcgaaagcctgacggagcaacgccgcgtgagtgatgaaggtcttcggatcgtaaaactctgttattagggaagaacatacgtgtaagtaactatgcacgtcttgacggtacctaatcagaaagccacggctaactacgtgccagcagccgcggtaatacgtaggtggcaagcgttatccggaattattgggcgtaaagcgcgcgtaggcggttttttaagtctgatgtgaaagcccacggctcaaccgtggagggtcattggaaactggaaaacttgagtgcagaagaggaaagtggaattccatgtgtagcggtgaaatgcgcagagatatggaggaacaccagtggcgaaggcgactttctggtctgtaactgacgctgatgtgcgaaagcgtggggatcaaacaggattagataccctggtagtccacgccgtaaacgatgagtgctaagtgttagggggtttccgccccttagtgctgcagctaacgcattaagcactccgcctggggagtacgaccgcaaggttgaaactcaaaggaattgacggggacccgcacaagcggtggagcatgtggtttaattcgaagcaacgcgaagaaccttaccaaatcttgacatcctttgacaactctagagatagagccttccccttcgggggacaaagtgacaggtggtgcatggttgtcgtcagctcgtgtcgtgagatgttgggttaagtcccgcaacgagcgcaacccttaagcttagttgccatcattaagttgggcactctaagttgactgccggtgacaaaccggaggaaggtggggatgacgtcaaatcatcatgccccttatgatttgggctacacacgtgctacaatggacaatacaaagggcagcgaaaccgcgaggtcaagcaaatcccataaagttgttctcagttcggattgtagtctgcaactcgactacatgaagctgg

SEQ ID NO: 11 - DNA, 1268 bp, Staphylococcus haemolyticus
  source 1..1268: mol_type = genomic DNA
agcttgctcctttgacgttagcggcggacgggtgagtaacacgtgggtaacctacctataagactgggataacttcgggaaaccggagctaatactggataatatttcgaaccgcatggttcgatagtgaaagatggttttgctatcacttatagatggacccgcgccgtattagctagttggtaaggtaacggcttaccaaggcgacgatacgtagccgacctgagagggtgatcggccacactggaactgagacacggtccagactcctacgggaggcagcagtagggaatcttccgcaatgggcgaaagcctgacggagcaacgccgcgtgagtgatgaaggtcttcggatcgtaaaactctgttattagggaagaacatacgtgtaagtaactatgcacgtcttgacggtacctaatcagaaagccacggctaactacgtgccagcagccgcggtaatacgtaggtggcaagcgttatccggaattattgggcgtaaagcgcgcgtaggcggttttttaagtctgatgtgaaagcccacggctcaaccgtggagggtcattggaaactggaaaacttgagtgcagaagaggaaagtggaattccatgtgtagcggtgaaatgcgcagagatatggaggaacaccagtggcgaaggcgactttctggtctgtaactgacgctgatgtgcgaaagcgtggggatcaaacaggattagataccctggtagtccacgccgtaaacgatgagtgctaagtgttagggggtttccgccccttagtgctgcagctaacgcattaagcactccgcctggggagtacgaccgcaaggttgaaactcaaaggaattgacggggacccgcacaagcggtggagcatgtggtttaattcgaagcaacgcgaagaaccttaccaaatcttgacatcctttgacaactctagagatagagccttccccttcgggggacaaagtgacaggtggtgcatggttgtcgtcagctcgtgtcgtgagatgttgggttaagtcccgcaacgagcgcaacccttaagcttagttgccatcattaagttgggcactctaagttgactgccggtgacaaaccggaggaaggtggggatgacgtcaaatcatcatgccccttatgatttgggctacacacgtgctacaatggacaatacaaagggcagcgaaaccgcgaggtcaagcaaatcccataaagttgttctcagttcggattgtagtctgcaactcgactacatgaagctgg

SEQ ID NO: 12 - DNA, 1268 bp, Staphylococcus haemolyticus
  source 1..1268: mol_type = genomic DNA
agcttgctcctttgacgttagcggcggacgggtgagtaacacgtgggtaacctacctataagactgggataacttcgggaaaccggagctaataccggataatatttcaaaccgcatggttcgatagtgaaagatggttttgctatcacttatagatggacccgcgccgtattagctagttggtaaggtaacggcttaccaaggcgacgatacgtagccgacctgagagggtgatcggccacactggaactgagacacggtccagactcctacgggaggcagcagtagggaatcttccgcaatgggcgaaagcctgacggagcaacgccgcgtgagtgatgaaggtcttcggatcgtaaaactctgttattagggaagaacatacgtgtaagtaactatgcacgtcttgacggtacctaatcagaaagccacggctaactacgtgccagcagccgcggtaatacgtaggtggcaagcgttatccggaattattgggcgtaaagcgcgcgtaggcggttttttaagtctgatgtgaaagcccacggctcaaccgtggagggtcattggaaactggaaaacttgagtgcagaagaggaaagtggaattccatgtgtagcggtgaaatgcgcagagatatggaggaacaccagtggcgaaggcgactttctggtctgtaactgacgctgatgtgcgaaagcgtggggatcaaacaggattagataccctggtagtccacgccgtaaacgatgagtgctaagtgttagggggtttccgccccttagtgctgcagctaacgcattaagcactccgcctggggagtacgaccgcaaggttgaaactcaaaggaattgacggggacccgcacaagcggtggagcatgtggtttaattcgaagcaacgcgaagaaccttaccaaatcttgacatcctttgacaactctagagatagagccttccccttcgggggacaaagtgacaggtggtgcatggttgtcgtcagctcgtgtcgtgagatgttgggttaagtcccgcaacgagcgcaacccttaagcttagttgccatcattaagttgggcactctaagttgactgccggtgacaaaccggaggaaggtggggatgacgtcaaatcatcatgccccttatgatttgggctacacacgtgctacaatggacaatacaaagggcagcgaaaccgcgaggtcaagcaaatcccataaagttgttctcagttcggattgtagtctgcaactcgactacatgaagctgg

SEQ ID NO: 13 - DNA, 1268 bp, Staphylococcus haemolyticus
  source 1..1268: mol_type = genomic DNA
agcttgctcctttgacgttagcggcggacgggtgagtaacacgtgggtaacctacctataagactgggataacttcgggaaaccggagctaataccggataatatttcgaaccgcatggttcgatagtgaaagatggttttgctatcacttatagatggacccgcgccgtattagctagttggtaaggtaacggcttaccaaggcgacgatacgtagccgacctgagagggtgatcggccacactggaactgagacacggtccagactcctacgggaggcagcagtagggaatcttccgcaatgggcgaaagcctgacggagcaacgccgcgtgagtgatgaaggtcttcggatcgtaaaactctgttattagggaagaacatacgtgtaagtaactgtgcacgtcttgacggtacctaatcagaaagccacggctaactacgtgccagcagccgcggtaatacgtaggtggcaagcgttatccggaattattgggcgtaaagcgcgcgtaggcggttttttaagtctgatgtgaaagcccacggctcaaccgtggagggtcattggaaactggaaaacttgagtgcagaagaggaaagtggaattccatgtgtagcggtgaaatgcgcagagatatggaggaacaccagtggcgaaggcgactttctggtctgtaactgacgctgatgtgcgaaagcgtggggatcaaacaggattagataccctggtagtccacgccgtaaacgatgagtgctaagtgttagggggtttccgccccttagtgctgcagctaacgcattaagcactccgcctggggagtacgaccgcaaggttgaaactcaaaggaattgacggggacccgcacaagcggtggagcatgtggtttaattcgaagcaacgcgaagaaccttaccaaatcttgacatcctttgacaactctagagatagagctttccccttcgggggacaaagtgacaggtggtgcatggttgtcgtcagctcgtgtcgtgagatgttgggttaagtcccgcaacgagcgcaacccttaagcttagttgccatcattaagttgggcactctaagttgactgccggtgacaaaccggaggaaggtggggatgacgtcaaatcatcatgccccttatgatttgggctacacacgtgctacaatggacaatacaaagggcagcgaaaccgcgaggtcaagcaaatcccataaagttgttctcagttcggattgtagtctgcaactcgactacatgaagctgg

SEQ ID NO: 14 - DNA, 1268 bp, Staphylococcus haemolyticus
  source 1..1268: mol_type = genomic DNA
agcttgctcctttgacgttagcggcggacgggtgagtaacacgtgggtaacctacctataagactgggataacttcgggaaaccggagctaataccggataatatttcgaaccgcatggttcgatagtgaaagatggttttgctatcacttatagatggacccgcgccgtattagctagttggtaaggtaacggcttaccaaggcgacgatacgtagccgacctgagagggtgatcggccacactggaactgagacacggtccagactcctacgggaggcagcagtagggaatcttccgcaatgggcgaaagcctgacggagcaacgccgcgtgagtgatgaaggtcttcggatcgtaaaactctgttattagggaagaacatacgtgtaagtaactgtgcacgtcttgacggtacctaatcagaaagccacggctaactacgtgccagcagccgcggtaatacgtaggtggcaagcgttatccggaattattgggcgtaaagcgcgcgtaggcggttttttaagtctgatgtgaaagcccacggctcaaccgtggagggtcattggaaactggaaaacttgagtgcagaagaggaaagtggaattccatgtgtagcggtgaaatgcgcagagatatggaggaacaccagtggcgaaggcgactttctggtctgtaactgacgctgatgtgcgaaagcgtggggatcaaacaggattagataccctggtagtccacgccgtaaacgatgagtgctaagtgttagggggtttccgccccttagtgctgcagctaacgcattaagcactccgcctggggagtacgaccgcaaggttgaaactcaaaggaattgacggggacccgcacaagcggtggagcatgtggtttaattcgaagcaacgcgaagaaccttaccaaatcttgacatcctttgacaactctagagatagagccttccccttcgggggacaaagtgacaggtggtgcatggttgtcgtcagctcgtgtcgtgagatgttgggttaagtcccgcaacgagcgcaacccttaagcttagttgccatcattaagttgggcactctaagttgactgccggtgacaaaccggaggaaggtggggatgacgtcaaatcatcatgccccttatgatttgggctacacacgtgctacaatggacaatacaaagggcagcgaaaccgcgaggtcaagcaaatcccataaagttgttctcagttcggattgtagtctgcaactcgactacatgaagctgg

SEQ ID NO: 15 - DNA, 1268 bp, Staphylococcus haemolyticus
  source 1..1268: mol_type = genomic DNA
agcttgctcctttgacgttagcggcggacgggtgagtaacacgtgggtaacctacctataagactgggataacttcgggaaaccggagctaataccggataatatttcgaaccgcatggttcgatagtgaaagatggttttgctatcacttatagatggacccgcgccgtattagctagttggtaaggtaacggcttaccaaggcgacgatacgtagccgacctgagagggtgatcggccacactggaactgagacacggtccagactcctacgggaggcagcagtagggaatcttccgcaatgggcgaaagcctgacggagcaacgccgcgtgagtgatgaaggtcttcggatcgtaaaactctgttattagggaagaacatacgtgtaagtaactgtgcacgtcttgacggtacctaatcagaaagccacggctaactacgtgccagcagccgcggtaatacgtaggtggcaagcgttatccggaattattgggcgtaaagcgcgcgtaggcggttttttaagtctgatgtgaaagcccacggctcaaccgtggagggtcattggaaactggaaaacttgagtgcagaagaggaaagtggaattccatgtgtagcggtgaaatgcgcagagatatggaggaacaccagtggcgaaggcgactttctggtctgtaactgacgctgatgtgcgaaagcgtggggatcaaacaggattagataccctggtagtccacgccgtaaacgatgagtgctaagtgttagggggtttccgccccttagtgctgcagctaacgcattaagcactccgcctggggagtacgaccgcaaggttgaaactcaaaggaattgacggggacccgcacaagcggtggagcatgtggtttaattcgaagcaacgcgaagaaccttaccaaatcttgacatcctttgacaactctagagatagagctttccccttcgggggacaaagtgacaggtggtgcatggttgtcgtcagctcgtgtcgtgagatgttgggttaagtcccgcaacgagcgcaacccttaagcttagttgccatcattaagttgggcactctaagttgactgccggtgacaaaccggaggaaggtggggatgacgtcaaatcatcatgccccttatgatttgggctacacacgtgctacaatggacaatacaaagggtagcgaaaccgcgaggtcaagcaaatcccataaagttgttctcagttcggattgtagtctgcaactcgactacatgaagctgg

SEQ ID NO: 16 - DNA, 1267 bp, Staphylococcus haemolyticus
  source 1..1267: mol_type = genomic DNA
agcttgctcctttgacgttagcggcggacgggtgagtaacacgtgggtaacctacctataagactgggataacttcgggaaaccggagctaataccggataatatttcgaaccgcatggttcgatagtgaaagatggttttgctatcacttatagatggacccgcgccgtattagctagttggtaaggtaacggcttaccaaggcgacgatacgtagccgacctgagagggtgatcggccacactggaactgagacacggtccagactcctacgggaggcagcagtagggaatcttccgcaatgggcgaaagcctgacggagcaacgccgcgtgagtgatgaaggtcttcggatcgtaaaactctgttattagggaagaacatacgtgtaagtaactgtgcacgtcttgacggtacctaatcagaaagccacggctaactacgtgccagcagccgcggtaatacgtaggtggcaagcgttatccggaattattgggcgtaaagcgcgcgtaggcggttttttaagtctgatgtgaaagcccacggctcaaccgtggagggtcattggaaactggaaaacttgagtgcagaagaggaaagtggaattccatgtgtagcggtgaaatgcgcagagatatggaggaacaccagtggcgaaggcgactttctggtctgtaactgacgctgatgtgcgaaagcgtggggatcaaacaggattagataccctggtagtccacgccgtaaacgatgagtgctaagtgttagggggtttccgccccttagtgctgcagctaacgcattaagcactccgcctggggagtacgaccgcaaggttgaaactcaaaggaattgacggggacccgcacaagcggtggagcatgtggtttaattcgaagcaacgcgaagaaccttaccaaatcttgacatcctttgacaactctagagatagagctttccccttcgggggacaaagtgacaggtggtgcatggttgtcgtcagctcgtgtcgtgagatgttgggttaagtcccgcaacgagcgcaacccttaagcttagttgccatcattaagttgggcactctaagttgactgccggtgacaaaccggaggaaggtgggggatgacgtcaaatcatcatgccccttatgatttgggctacacacgtgctacaatggacaatacaaagggcagcgaaacccgcgaggtcaagcaatcccataagttgtctcagttcgggattgtagtctgcaactcgactacatgagctgg

SEQ ID NO: 17 - DNA, 1268 bp, Staphylococcus warneri
  source 1..1268: mol_type = genomic DNA
agcttgctcctttgacgttagcggcggacgggtgagtaacacgtggataacctacctataagactgggataacttcgggaaaccggagctaataccggataacatattgaaccgcatggttcaatagtgaaaggcggctttgctgtcacttatagatggatccgcgccgtattagctagttggtaaggtaacggcttaccaaggcaacgatacgtagccgacctgagagggtgatcggccacactggaactgagacacggtccagactcctacgggaggcagcagtagggaatcttccgcaatgggcgaaagcctgacggagcaacgccgcgtgagtgatgaaggtcttcggatcgtaaaactctgttatcagggaagaacaaatgtgtaagtaactgtgcacatcttgacggtacctgatcagaaagccacggctaactacgtgccagcagccgcggtaatacgtaggtggcaagcgttatccggaattattgggcgtaaagcgcgcgtaggcggttttttaagtctgatgtgaaagcccacggctcaaccgtggagggtcattggaaactggaaaacttgagtgcagaagaggaaagtggaattccatgtgtagcggtgaaatgcgcagagatatggaggaacaccagtggcgaaggcgactttctggtctgtaactgacgctgatgtgcgaaagcgtggggatcaaacaggattagataccctggtagtccacgccgtaaacgatgagtgctaagtgttagggggtttccgccccttagtgctgcagctaacgcattaagcactccgcctggggagtacgaccgcaaggttgaaactcaaaggaattgacggggacccgcacaagcggtggagcatgtggtttaattcgaagcaacgcgaagaaccttaccaaatcttgacatcctttgaccgctctagagatagagtcttccccttcgggggacaaagtgacaggtggtgcatggttgtcgtcagctcgtgtcgtgagatgttgggttaagtcccgcaacgagcgcaacccttaagcttagttgccatcattaagttgggcactctaagttgactgccggtgacaaaccggaggaaggtggggatgacgtcaaatcatcatgccccttatgatttgggctacacacgtgctacaatggacaatacaaagggcagctaaaccgcgaggtcaagcaaatcccataaagttgttctcagttcggattgtagtctgcaactcgactacatgaagctgg

SEQ ID NO: 18 - DNA, 1268 bp, Staphylococcus warneri
  source 1..1268: mol_type = genomic DNA
agcttgctcctttgacgttagcggcggacgggtgagtaacacgtggataacgtacctataagactgggataacttcgggaaaccggagctaataccggataacatattgaaccgcatggttcaatagtgaaaggcggctttgctgtcacttatagatggatccgcgccgtattagctagttggtaaggtaacggcttaccaaggcaacgatacgtagccgacctgagagggtgatcggccacactggaactgagacacggtccagactcctacgggaggcagcagtagggaatcttccgcaatgggcgaaagcctgacggagcaacgccgcgtgagtgatgaaggtcttcggatcgtaaaactctgttatcagggaagaacaaatgtgtaagtaactgtgcacatcttgacggtacctgatcagaaagccacggctaactacgtgccagcagccgcggtaatacgtaggtggcaagcgttatccggaattattgggcgtaaagcgcgcgtaggcggttttttaagtctgatgtgaaagcccacggctcaaccgtggagggtcattggaaactggaaaacttgagtgcagaagaggaaagtggaattccatgtgtagcggtgaaatgcgcagagatatggaggaacaccagtggcgaaggcgactttctggtctgtaactgacgctgatgtgcgaaagcgtggggatcaaacaggattagataccctggtagtccacgccgtaaacgatgagtgctaagtgttagggggtttccgccccttagtgctgcagctaacgcattaagcactccgcctggggagtacgaccgcaaggttgaaactcaaaggaattgacggggacccgcacaagcggtggagcatgtggtttaattcgaagcaacgcgaagaaccttaccaaatcttgacatcctttgaccgctctagagatagagtcttccccttcgggggacaaagtgacaggtggtgcatggttgtcgtcagctcgtgtcgtgagatgttgggttaagtcccgcaacgagcgcaacccttaagcttagttgccatcattaagttgggcactctaagttgactgccggtgacaaaccggaggaaggtggggatgacgtcaaatcatcatgccccttatgatttgggctacacacgtgctacaatggacaatacaaagggcagctaaaccgcgaggtcaagcaaatcccataaagttgttctcagttcggattgtagtctgcaactcgactacatgaagctgg

SEQ ID NO: 19 - DNA, 16 bp, synthetic construct
  source 1..16: mol_type = other DNA; note = forward primer F1
gtttgatcctggctca

SEQ ID NO: 20 - DNA, 16 bp, synthetic construct
  source 1..16: mol_type = other DNA; note = reverse primer R2
taccttgttacgactt

SEQ ID NO: 21 - DNA, 18 bp, synthetic construct
  source 1..18: mol_type = other DNA; note = forward primer F2
ggattagataccctggta